European Patent Specification EP 3 470 395 B1, published September 2, 2026. Title: AMINE-CONTAINING TRANSFECTION REAGENTS AND METHODS FOR MAKING AND USING SAME. Applicant: YANG, ZHIWEI ANGRISH, PARUL DE MOLLERAT DU JEU, XAVIER WIEDERHOLT, KRISTIN. Application 13/297,231. The sequence listing filed with the application follows.

SEQUENCE LISTING (4 sequences)

SEQ ID NO: 1 - RNA, 25 nt, Artificial Sequence
  Description of Artificial Sequence: Synthetic oligonucleotide
auuugcacagaucagcugcucauuc

SEQ ID NO: 2 - RNA, 21 nt, Artificial Sequence
  Description of Artificial Sequence: Synthetic oligonucleotide
aaacuauaaucguacaucuga

SEQ ID NO: 3 - DNA, 21 bp, Artificial Sequence
  Description of Artificial Sequence: Synthetic oligonucleotide
  Description of Combined DNA/RNA Molecule: Synthetic oligonucleotide
uuacgucgucgcgucguuatt

SEQ ID NO: 4 - DNA, 1750 bp, Artificial Sequence
  Description of Artificial Sequence: Synthetic polynucleotide
ttggaccctcgtacagaagctaatacgactcactatatgggcggtaggcgtgtacggtgggaggtctatataagcagagctcgcaacttttctatacaaagttgctatgggcccaaagaagaagagaaaggtttcgaatttactgaccgtacaccaaaatttgcctgcattaccggtcgatgcaacgagtgatgaggttcgcaagaacctgatggacatgttcagggatcgccaggcgttttctgagcatacctggaaaatgcttctgtccgtttgccggtcgtgggcggcatggtgcaagttgaataaccggaaatggtttcccgcagaacctgaagatgttcgcgattatcttctatatcttcaggcgcgcggtctggcagtaaaaactatccagcaacatttgggccagctaaacatgcttcatcgtcggtccgggctgccacgaccaagtgacagcaatgctgtttcactggttatgcggcggatccgaaaagaaaacgttgatgccggtgaacgtgcaaaacaggctctagcgttcgaacgcactgatttcgaccaggttcgttcactcatggaaaatagcgatcgctgccaggatatacgtaatctggcatttctggggattgcttataacaccctgttacgtatagccgaaattgccaggatcagggttaaagatatctcacgtactgacggtgggagaatgttaatccatattggcagaacgaaaacgctggttagcaccgcaggtgtagagaaggcacttagcctgggggtaactaaactggtcgagcgatggatttccgtctctggtgtagctgatgatccgaataactacctgttttgccgggtcagaaaaaatggtgttgccgcgccatctgccaccagccagctatcaactcgcgccctggaagggatttttgaagcaactcatcgattgatttacggcgctaaggatgactctggtcagagatacctggcctggtctggacacagtgcccgtgtcggagccgcgcgagatatggcccgcgctggagtttcaataccggagatcatgcaagctggtggctggaccaatgtaaatattgtcatgaactatatccgtaacctggatagtgaaacaggggcaatggtgcgcctgctggaagatggcgattagacatagcagcaattggcaagctgcttatatagaacttgcggcgattggcatgccgctttaaaattttattttattttcttttcttttccgaatcggatacatagcagcaattggcaagctgcttatatagaacttgcggcgattggcatgccgctttaaaattttattttattttcttttcttttccgaatcggatacatagcagcaattggcaagctgcttatatagaacttgcggcgattggcatgccgctttaaaattttattttattttcttttcttttccgaatcggatacatagcagcaattggcaagctgcttatatagaacttgcggcgattggcatgccgctttaaaattttattttattttcttttcttttccgaatcggatacatagcagcaattggcaagctgcttatatagaacttgcggcgattggcatgccgctttaaaattttattttattttcttttcttttccgaatcggatacatagcagcaattggcaagctgcttatatagaacttgcggcgattggcatgccgctttaaaattttattttattttcttttcttttccgaatcggat